European Patent Application EP 4 588 521 A2, published July 23, 2025. Title: POLYPEPTIDE-ANTIGEN CONJUGATES WITH NON-NATURAL AMINO ACIDS. Applicant: Vaxcyte, Inc. Application WO PCT/US2017/069129, filed December 29, 2017. The sequence listing filed with the application follows.

SEQUENCE LISTING (10 sequences)

SEQ ID NO: 1 - protein, 536 aa, Corynebacterium diphtheriae
MGADDVVDSSKSFVMENFSSYHGTKPGYVDSIQKGIQKPKSGTQGNYDDDWKEFYSTDNKYDAAGYSVDNENPLSGKAGGVVKVTYPGLTKVLALKVDNAETIKKELGLSLTEPLMEQVGTEEFIKRFGDGASRVVLSLPFAEGSSSVEYINNWEQAKALSVELEINFETRGKRGQDAMYEYMAQACAGNRVRRSVGSSLSCINLDWDVIRDKTKTKIESLKEHGPIKNKMSESPNKTVSEEKAKQYLEEFHQTALEHPELSELKTVTGTNPVFAGANYAAWAVNVAQVIDSETADNLEKTTAALSILPGIGSVMGIADGAVHHNTEEIVAQSIALSSLMVAQAIPLVGELVDIGFAAYNFVESIINLFQVVHNSYNRPAYSPGHKTQPFLHDGYAVSWNTVEDSIIRTGFQGESGHDIKITAENTPLPIAGVLLPTIPGKLDVNKSKTHISVNGRKIRMRCRAIDGDVTFCRPKSPVYVGNGVHANLHVAFHRSSSEKIHSNEISSDSIGVLGYQKTVDHTKVNSKLSLFFEIKS

SEQ ID NO: 2 - DNA, 1611 bp, Corynebacterium diphtheriae
  source 1..1611: mol_type = other DNA
atgggcgcagacgatgttgtggactcaagtaaatcatttgtcatggaaaacttctcctcatatcacggcacgaaaccgggctacgttgatagcattcagaaaggtatccaaaaaccgaaatctggcacgcagggtaactacgatgacgattggaaagaattctacagcaccgacaacaaatatgatgcggccggttactcagtcgacaacgaaaatccgctgtcgggcaaagccggcggtgtggttaaagtgacgtatccgggcctgaccaaagtcctggccctgaaagtggataatgcagaaaccatcaaaaaagaactgggtctgagcctgacggaaccgctgatggaacaggttggcaccgaagaatttatcaaacgcttcggcgatggtgccagtcgtgtcgtgctgtccctgccgttcgcagaaggtagctctagtgtggaatatattaacaattgggaacaagcgaaagccctgtccgttgaactggaaatcaactttgaaacccgcggcaaacgtggtcaggatgcgatgtatgaatacatggcacaagcttgcgcgggtaatcgcgttcgtcgcagcgtcggctcctcactgtcttgtatcaacctggactgggatgttatccgtgataaaaccaaaacgaaaatcgaaagtctgaaagaacatggcccgatcaaaaacaaaatgagcgaatctccgaataaaacggtgtccgaagaaaaagctaaacagtatctggaagaattccaccaaaccgcactggaacatccggaactgtcagaactgaaaaccgtgacgggtaccaacccggtttttgccggcgcaaattacgcagcttgggctgtgaacgttgcgcaagtgattgactcggaaacggccgataatctggaaaaaaccacggcggccctgagtattctgccgggcatcggttccgttatgggtattgccgacggcgcagtccatcacaacaccgaagaaattgtggcccagtctatcgcactgtcgagcctgatggttgctcaagcgattccgctggttggcgaactggttgatatcggctttgcagcttacaacttcgtggaaagtattatcaacctgtttcaggttgtccacaactcatataatcgcccggcctactcgccgggtcacaaaacccaaccgttcctgcatgacggctacgcggttagctggaatacggtcgaagattctattatccgtaccggctttcagggtgaatctggccacgacattaaaatcacggctgaaaacaccccgctgccgattgcaggtgttctgctgccgacgatcccgggtaaactggatgttaacaaatcaaaaacccatatctcggtcaacggtcgcaaaattcgtatgcgctgccgtgcgatcgacggcgatgtgaccttctgtcgtccgaaaagcccggtctatgtgggcaacggtgtccatgctaatctgcacgtggcgtttcatcgctctagttccgaaaaaatccatagtaacgaaatctcatcggattccattggtgtgctgggctaccagaaaaccgtggaccataccaaagtgaatagcaaactgagcctgttcttcgaaatcaaatcgtaa

SEQ ID NO: 3 - protein, 19 aa, Clostridium tetani
DKISDVSTIVPYIGPALNI

SEQ ID NO: 4 - protein, 20 aa, Clostridium tetani
NNFTVSFWLRVPKVSASHLE

SEQ ID NO: 5 - protein, 16 aa, Streptococcus G148
VSDYYKNLINNAKTVE

SEQ ID NO: 6 - protein, 16 aa, Streptococcus G148
DGLSDFLKSQTPAEDT

SEQ ID NO: 7 - protein, 16 aa, Streptococcus G148
AEDTVKSIELAEAKVL

SEQ ID NO: 8 - protein, 346 aa, Haemophilus influenzae
CSSHSSNMANTQMKSDKIIIAHRGASGYLPEHTLESKALAFAQQADYLEQDLAMTKDGRLVVIHDHFLDGLTDVAKKFPHRHRKDGRYYVIDFTLKEIQSLEMTENFETKDGKQAQVYPNRFPLWKSHFRIHTFEDEIEFIQGLEKSTGKKVGIYPEIKAPWFHHQNGKDIAAETLKVLKKYGYDKKTDMVYLQTFDFNELKRIKTELLPQMGMDLKLVQLIAYTDWKETQEKDPKGYWVNYNYDWMFKPGAMAEVVKYADGVGPGWYMLVNKEESKPDNIVYTPLVKELAQYNVEVHPYTVRKDALPEFFTDVNQMYDALLNKSGATGVFTDFPDTGVEFLKGIK

SEQ ID NO: 9 - protein, 536 aa, synthetic construct
  REGION 1..536: note = Modified carrier protein
  MOD_RES 34: note = Xaa is a non-natural amino acid
  MOD_RES 213: note = Xaa is a non-natural amino acid
  MOD_RES 245: note = Xaa is a non-natural amino acid
  MOD_RES 265: note = Xaa is a non-natural amino acid
  MOD_RES 386: note = Xaa is a non-natural amino acid
  MOD_RES 527: note = Xaa is a non-natural amino acid
MGADDVVDSSKSFVMENFSSYHGTKPGYVDSIQXGIQKPKSGTQGNYDDDWKEFYSTDNKYDAAGYSVDNENPLSGKAGGVVKVTYPGLTKVLALKVDNAETIKKELGLSLTEPLMEQVGTEEFIKRFGDGASRVVLSLPFAEGSSSVEYINNWEQAKALSVELEINFETRGKRGQDAMYEYMAQACAGNRVRRSVGSSLSCINLDWDVIRDXTKTKIESLKEHGPIKNKMSESPNKTVSEEKAXQYLEEFHQTALEHPELSELXTVTGTNPVFAGANYAAWAVNVAQVIDSETADNLEKTTAALSILPGIGSVMGIADGAVHHNTEEIVAQSIALSSLMVAQAIPLVGELVDIGFAAYNFVESIINLFQVVHNSYNRPAYSPGHXTQPFLHDGYAVSWNTVEDSIIRTGFQGESGHDIKITAENTPLPIAGVLLPTIPGKLDVNKSKTHISVNGRKIRMRCRAIDGDVTFCRPKSPVYVGNGVHANLHVAFHRSSSEKIHSNEISSDSIGVLGYQKTVDHTKVNSXLSLFFEIKS

SEQ ID NO: 10 - protein, 9 aa, synthetic construct
  REGION 1..9: note = Histidine tag
GSGHHHHHH